European Patent Application EP 4 768 919 A1, published July 1, 2026. Title: USE OF N-TERMINAL FRAGMENT OF IGFBP-4 IN CLINICAL ASSESSMENT OF HEART FAILURE AND CORONARY HEART DISEASE. Applicant: SHENZHEN MINDRAY BIO MEDICAL ELECTRONICS CO LTD. The sequence listing filed with the application follows.

SEQUENCE LISTING (1 sequence)

SEQ ID NO: 1 - protein, 135 aa, synthetic construct
DEAIHCPPCSEEKLARCRPPVGCEELVREPGCGCCATCALGLGMPCGVYTPRCGSGLRCYPPRGVEKPLHTLMHGQGVCMELAEIEAIQESLQPSDKDEGDHPNNSFSPCSAHDRRCLQKHFAKIRDRSTSGGKM